European Patent Specification EP 3 564 255 B1, published April 8, 2026. Title: Dual functional peptide for cell penetration and bone tissue regeneration and use of the same. Applicant: NANO INTELLIGENT BIOMEDICAL ENGINEERING CORPORATION. CO. LTD SEOUL NATIONAL UNIVERSITY R&DB FOUNDATION. The sequence listing filed with the application follows.

SEQUENCE LISTING (6 sequences)

SEQ ID NO: 1 - protein, 10 aa, Artificial Sequence
  Dual functional candidate peptide for cell penetration and bone tissue regeneration
STTFEEMQKA

SEQ ID NO: 2 - protein, 10 aa, Artificial Sequence
  Dual functional candidate peptide for cell penetration and bone tissue regeneration
FEEGQAQWDC

SEQ ID NO: 3 - protein, 20 aa, Artificial Sequence
  Dual functional candidate peptide for cell penetration and bone tissue regeneration
FEEGQAQWDCVNPKYKQKRR

SEQ ID NO: 4 - protein, 10 aa, Artificial Sequence
  Dual functional peptide for cell penetration and bone tissue regeneration
VNPKYKQKRR

SEQ ID NO: 5 - protein, 10 aa, Artificial Sequence
  Dual functional candidate peptide for cell penetration and bone tissue regeneration
SYKNSGVVVL

SEQ ID NO: 6 - protein, 20 aa, Artificial Sequence
  Dual functional candidate peptide for cell penetration and bone tissue regeneration
VNPKYKQKRRSYKNSGVVVL